European Patent Application EP 4 706 637 A1, published March 11, 2026. Title: DRUG FOR GENETIC MODIFICATION, DRUG DELIVERY METHOD, AND DRUG DELIVERY CARRIER. Applicant: Kabushiki Kaisha Toshiba. Application EP. The sequence listing filed with the application follows.

SEQUENCE LISTING (8 sequences)

SEQ ID NO: 1 - protein, 20 aa, synthetic construct
RQRQRYYRQRQRGGRRRRRR

SEQ ID NO: 2 - protein, 13 aa, synthetic construct
RQRQRGGRRRRRR

SEQ ID NO: 3 - protein, 21 aa, synthetic construct
RRRRRRYYRQRQRGGRRRRRR

SEQ ID NO: 4 - protein, 39 aa, synthetic construct
GNQSSNFGPMKGGNFGGRSSGPYGGGGQYFAKPRNQGGY

SEQ ID NO: 5 - RNA, 4448 nt, synthetic construct
  source 1..4448: mol_type = other RNA
aggaataaactagtattcttctggtccccacagactcagagagaacccgccaccatggccaccatggactataaggaccacgacggagactacaaggatcatgatattgattacaaagacgatgacgataagatggccccaaagaagaagcggaaggtcggtatccacggagtcccagcagccgacaagaagtacagcatcggcctggacatcggcaccaactctgtgggctgggccgtgatcaccgacgagtacaaggtgcccagcaagaaattcaaggtgctgggcaacaccgaccggcacagcatcaagaagaacctgatcggagccctgctgttcgacagcggcgaaacagccgaggccacccggctgaagagaaccgccagaagaagatacaccagacggaagaaccggatctgctatctgcaagagatcttcagcaacgagatggccaaggtggacgacagcttcttccacagactggaagagtccttcctggtggaagaggataagaagcacgagcggcaccccatcttcggcaacatcgtggacgaggtggcctaccacgagaagtaccccaccatctaccacctgagaaagaaactggtggacagcaccgacaaggccgacctgcggctgatctatctggccctggcccacatgatcaagttccggggccacttcctgatcgagggcgacctgaaccccgacaacagcgacgtggacaagctgttcatccagctggtgcagacctacaaccagctgttcgaggaaaaccccatcaacgccagcggcgtggacgccaaggccatcctgtctgccagactgagcaagagcagacggctggaaaatctgatcgcccagctgcccggcgagaagaagaatggcctgttcggaaacctgattgccctgagcctgggcctgacccccaacttcaagagcaacttcgacctggccgaggatgccaaactgcagctgagcaaggacacctacgacgacgacctggacaacctgctggcccagatcggcgaccagtacgccgacctgtttctggccgccaagaacctgtccgacgccatcctgctgagcgacatcctgagagtgaacaccgagatcaccaaggcccccctgagcgcctctatgatcaagagatacgacgagcaccaccaggacctgaccctgctgaaagctctcgtgcggcagcagctgcctgagaagtacaaagagattttcttcgaccagagcaagaacggctacgccggctacattgacggcggagccagccaggaagagttctacaagttcatcaagcccatcctggaaaagatggacggcaccgaggaactgctcgtgaagctgaacagagaggacctgctgcggaagcagcggaccttcgacaacggcagcatcccccaccagatccacctgggagagctgcacgccattctgcggcggcaggaagatttttacccattcctgaaggacaaccgggaaaagatcgagaagatcctgaccttccgcatcccctactacgtgggccctctggccaggggaaacagcagattcgcctggatgaccagaaagagcgaggaaaccatcaccccctggaacttcgaggaagtggtggacaagggcgcttccgcccagagcttcatcgagcggatgaccaacttcgataagaacctgcccaacgagaaggtgctgcccaagcacagcctgctgtacgagtacttcaccgtgtataacgagctgaccaaagtgaaatacgtgaccgagggaatgagaaagcccgccttcctgagcggcgagcagaaaaaggccatcgtggacctgctgttcaagaccaaccggaaagtgaccgtgaagcagctgaaagaggactacttcaagaaaatcgagtgcttcgactccgtggaaatctccggcgtggaagatcggttcaacgcctccctgggcacataccacgatctgctgaaaattatcaaggacaaggacttcctggacaatgaggaaaacgaggacattctggaagatatcgtgctgaccctgacactgtttgaggacagagagatgatcgaggaacggctgaaaacctatgcccacctgttcgacgacaaagtgatgaagcagctgaagcggcggagatacaccggctggggcaggctgagccggaagctgatcaacggcatccgggacaagcagtccggcaagacaatcctggatttcctgaagtccgacggcttcgccaacagaaacttcatgcagctgatccacgacgacagcctgacctttaaagaggacatccagaaagcccaggtgtccggccagggcgatagcctgcacgagcacattgccaatctggccggcagccccgccattaagaagggcatcctgcagacagtgaaggtggtggacgagctcgtgaaagtgatgggccggcacaagcccgagaacatcgtgatcgaaatggccagagagaaccagaccacccagaagggacagaagaacagccgcgagagaatgaagcggatcgaagagggcatcaaagagctgggcagccagatcctgaaagaacaccccgtggaaaacacccagctgcagaacgagaagctgtacctgtactacctgcagaatgggcgggatatgtacgtggaccaggaactggacatcaaccggctgtccgactacgatgtggaccatatcgtgcctcagagctttctgaaggacgactccatcgacaacaaggtgctgaccagaagcgacaagaaccggggcaagagcgacaacgtgccctccgaagaggtcgtgaagaagatgaagaactactggcggcagctgctgaacgccaagctgattacccagagaaagttcgacaatctgaccaaggccgagagaggcggcctgagcgaactggataaggccggcttcatcaagagacagctggtggaaacccggcagatcacaaagcacgtggcacagatcctggactcccggatgaacactaagtacgacgagaatgacaagctgatccgggaagtgaaagtgatcaccctgaagtccaagctggtgtccgatttccggaaggatttccagttttacaaagtgcgcgagatcaacaactaccaccacgcccacgacgcctacctgaacgccgtcgtgggaaccgccctgatcaaaaagtaccctaagctggaaagcgagttcgtgtacggcgactacaaggtgtacgacgtgcggaagatgatcgccaagagcgagcaggaaatcggcaaggctaccgccaagtacttcttctacagcaacatcatgaactttttcaagaccgagattaccctggccaacggcgagatccggaagcggcctctgatcgagacaaacggcgaaaccggggagatcgtgtgggataagggccgggattttgccaccgtgcggaaagtgctgagcatgccccaagtgaatatcgtgaaaaagaccgaggtgcagacaggcggcttcagcaaagagtctatcctgcccaagaggaacagcgataagctgatcgccagaaagaaggactgggaccctaagaagtacggcggcttcgacagccccaccgtggcctattctgtgctggtggtggccaaagtggaaaagggcaagtccaagaaactgaagagtgtgaaagagctgctggggatcaccatcatggaaagaagcagcttcgagaagaatcccatcgactttctggaagccaagggctacaaagaagtgaaaaaggacctgatcatcaagctgcctaagtactccctgttcgagctggaaaacggccggaagagaatgctggcctctgccggcgaactgcagaagggaaacgaactggccctgccctccaaatatgtgaacttcctgtacctggccagccactatgagaagctgaagggctcccccgaggataatgagcagaaacagctgtttgtggaacagcacaagcactacctggacgagatcatcgagcagatcagcgagttctccaagagagtgatcctggccgacgctaatctggacaaagtgctgtccgcctacaacaagcaccgggataagcccatcagagagcaggccgagaatatcatccacctgtttaccctgaccaatctgggagcccctgccgccttcaagtactttgacaccaccatcgaccggaagaggtacaccagcaccaaagaggtgctggacgccaccctgatccaccagagcatcaccggcctgtacgagacacggatcgacctgtctcagctgggaggcgacaaaaggccggcggccacgaaaaaggccggccaggcaaaaaagaaaaagtgatgagctggagcctcggtggcctagcttcttgccccttgggcctccccccagcccctcctccccttcctgcacccgtacccccgtggtctttgaataaagtctgagtgggcggc

SEQ ID NO: 6 - RNA, 5213 nt, synthetic construct
  source 1..5213: mol_type = other RNA
aggaataaactagtattcttctggtccccacagactcagagagaacccgccaccgccaccatggactataaggaccacgacggagactacaaggatcatgatattgattacaaagacgatgacgataagatggccccaaagaagaagcggaaggtcggtatccacggagtcccagcagccgacaagaagtacagcatcggcctggacatcggcaccaactctgtgggctgggccgtgatcaccgacgagtacaaggtgcccagcaagaaattcaaggtgctgggcaacaccgaccggcacagcatcaagaagaacctgatcggagccctgctgttcgacagcggcgaaacagccgaggccacccggctgaagagaaccgccagaagaagatacaccagacggaagaaccggatctgctatctgcaagagatcttcagcaacgagatggccaaggtggacgacagcttcttccacagactggaagagtccttcctggtggaagaggataagaagcacgagcggcaccccatcttcggcaacatcgtggacgaggtggcctaccacgagaagtaccccaccatctaccacctgagaaagaaactggtggacagcaccgacaaggccgacctgcggctgatctatctggccctggcccacatgatcaagttccggggccacttcctgatcgagggcgacctgaaccccgacaacagcgacgtggacaagctgttcatccagctggtgcagacctacaaccagctgttcgaggaaaaccccatcaacgccagcggcgtggacgccaaggccatcctgtctgccagactgagcaagagcagacggctggaaaatctgatcgcccagctgcccggcgagaagaagaatggcctgttcggaaacctgattgccctgagcctgggcctgacccccaacttcaagagcaacttcgacctggccgaggatgccaaactgcagctgagcaaggacacctacgacgacgacctggacaacctgctggcccagatcggcgaccagtacgccgacctgtttctggccgccaagaacctgtccgacgccatcctgctgagcgacatcctgagagtgaacaccgagatcaccaaggcccccctgagcgcctctatgatcaagagatacgacgagcaccaccaggacctgaccctgctgaaagctctcgtgcggcagcagctgcctgagaagtacaaagagattttcttcgaccagagcaagaacggctacgccggctacattgacggcggagccagccaggaagagttctacaagttcatcaagcccatcctggaaaagatggacggcaccgaggaactgctcgtgaagctgaacagagaggacctgctgcggaagcagcggaccttcgacaacggcagcatcccccaccagatccacctgggagagctgcacgccattctgcggcggcaggaagatttttacccattcctgaaggacaaccgggaaaagatcgagaagatcctgaccttccgcatcccctactacgtgggccctctggccaggggaaacagcagattcgcctggatgaccagaaagagcgaggaaaccatcaccccctggaacttcgaggaagtggtggacaagggcgcttccgcccagagcttcatcgagcggatgaccaacttcgataagaacctgcccaacgagaaggtgctgcccaagcacagcctgctgtacgagtacttcaccgtgtataacgagctgaccaaagtgaaatacgtgaccgagggaatgagaaagcccgccttcctgagcggcgagcagaaaaaggccatcgtggacctgctgttcaagaccaaccggaaagtgaccgtgaagcagctgaaagaggactacttcaagaaaatcgagtgcttcgactccgtggaaatctccggcgtggaagatcggttcaacgcctccctgggcacataccacgatctgctgaaaattatcaaggacaaggacttcctggacaatgaggaaaacgaggacattctggaagatatcgtgctgaccctgacactgtttgaggacagagagatgatcgaggaacggctgaaaacctatgcccacctgttcgacgacaaagtgatgaagcagctgaagcggcggagatacaccggctggggcaggctgagccggaagctgatcaacggcatccgggacaagcagtccggcaagacaatcctggatttcctgaagtccgacggcttcgccaacagaaacttcatgcagctgatccacgacgacagcctgacctttaaagaggacatccagaaagcccaggtgtccggccagggcgatagcctgcacgagcacattgccaatctggccggcagccccgccattaagaagggcatcctgcagacagtgaaggtggtggacgagctcgtgaaagtgatgggccggcacaagcccgagaacatcgtgatcgaaatggccagagagaaccagaccacccagaagggacagaagaacagccgcgagagaatgaagcggatcgaagagggcatcaaagagctgggcagccagatcctgaaagaacaccccgtggaaaacacccagctgcagaacgagaagctgtacctgtactacctgcagaatgggcgggatatgtacgtggaccaggaactggacatcaaccggctgtccgactacgatgtggaccatatcgtgcctcagagctttctgaaggacgactccatcgacaacaaggtgctgaccagaagcgacaagaaccggggcaagagcgacaacgtgccctccgaagaggtcgtgaagaagatgaagaactactggcggcagctgctgaacgccaagctgattacccagagaaagttcgacaatctgaccaaggccgagagaggcggcctgagcgaactggataaggccggcttcatcaagagacagctggtggaaacccggcagatcacaaagcacgtggcacagatcctggactcccggatgaacactaagtacgacgagaatgacaagctgatccgggaagtgaaagtgatcaccctgaagtccaagctggtgtccgatttccggaaggatttccagttttacaaagtgcgcgagatcaacaactaccaccacgcccacgacgcctacctgaacgccgtcgtgggaaccgccctgatcaaaaagtaccctaagctggaaagcgagttcgtgtacggcgactacaaggtgtacgacgtgcggaagatgatcgccaagagcgagcaggaaatcggcaaggctaccgccaagtacttcttctacagcaacatcatgaactttttcaagaccgagattaccctggccaacggcgagatccggaagcggcctctgatcgagacaaacggcgaaaccggggagatcgtgtgggataagggccgggattttgccaccgtgcggaaagtgctgagcatgccccaagtgaatatcgtgaaaaagaccgaggtgcagacaggcggcttcagcaaagagtctatcctgcccaagaggaacagcgataagctgatcgccagaaagaaggactgggaccctaagaagtacggcggcttcgacagccccaccgtggcctattctgtgctggtggtggccaaagtggaaaagggcaagtccaagaaactgaagagtgtgaaagagctgctggggatcaccatcatggaaagaagcagcttcgagaagaatcccatcgactttctggaagccaagggctacaaagaagtgaaaaaggacctgatcatcaagctgcctaagtactccctgttcgagctggaaaacggccggaagagaatgctggcctctgccggcgaactgcagaagggaaacgaactggccctgccctccaaatatgtgaacttcctgtacctggccagccactatgagaagctgaagggctcccccgaggataatgagcagaaacagctgtttgtggaacagcacaagcactacctggacgagatcatcgagcagatcagcgagttctccaagagagtgatcctggccgacgctaatctggacaaagtgctgtccgcctacaacaagcaccgggataagcccatcagagagcaggccgagaatatcatccacctgtttaccctgaccaatctgggagcccctgccgccttcaagtactttgacaccaccatcgaccggaagaggtacaccagcaccaaagaggtgctggacgccaccctgatccaccagagcatcaccggcctgtacgagacacggatcgacctgtctcagctgggaggcgacaaaaggccggcggccacgaaaaaggccggccaggcaaaaaagaaaaagggcggtgagggcagaggaagtctgctaacatgcggtgacgtcgaggagaatcctggcccaatggtgagcaagggcgaggaggataacatggccatcatcaaggagttcatgcgcttcaaggtgcacatggagggctccgtgaacggccacgagttcgagatcgagggcgagggcgagggccgcccctacgagggcacccagaccgccaagctgaaggtgaccaagggtggccccctgcccttcgcctgggacatcctgtcccctcagttcatgtacggctccaaggcctacgtgaagcaccccgccgacatccccgactacttgaagctgtccttccccgagggcttcaagtgggagcgcgtgatgaacttcgaggacggcggcgtggtgaccgtgacccaggactcctccctgcaggacggcgagttcatctacaaggtgaagctgcgcggcaccaacttcccctccgacggccccgtaatgcagaagaagaccatgggctgggaggcctcctccgagcggatgtaccccgaggacggcgccctgaagggcgagatcaagcagaggctgaagctgaaggacggcggccactacgacgctgaggtcaagaccacctacaaggccaagaagcccgtgcagctgcccggcgcctacaacgtcaacatcaagttggacatcacctcccacaacgaggactacaccatcgtggaacagtacgaacgcgccgagggccgccactccaccggcggcatggacgagctgtacaagtagtgagctggagcctcggtggcctagcttcttgccccttgggcctccccccagcccctcctccccttcctgcacccgtacccccgtggtctttgaataaagtctgagtgggcggc

SEQ ID NO: 7 - RNA, 20 nt, synthetic construct
  source 1..20: mol_type = other RNA
cgctatctgagcagcgctca

SEQ ID NO: 8 - RNA, 20 nt, synthetic construct
  source 1..20: mol_type = other RNA
ctcggataagatgctgagga